European Patent Application EP 4 574 845 A1, published June 25, 2025. Title: IL-15 MUTANT-Fc/IL-15Rα SUBUNIT-Fc HETERODIMER AND USE THEREOF. Applicant: HI-Lab (Beijing) Biotech. Co., Ltd. The sequence listing filed with the application follows.

SEQUENCE LISTING (40 sequences)

SEQ ID NO: 1 - protein, 114 aa, synthetic construct
NWVNVISDLKKIEDLIQSMHIDATLYTESDVHPSCKVTAMKCFLLELQVISLESGDASIHDTVENLIILANNSLSSNGNVTESGCKECEELEEKNIKEFLQSFVHIVQMFINTS

SEQ ID NO: 2 - protein, 78 aa, synthetic construct
ITCPPPMSVEHADIWVKSYSLYSRERYICNSGFKRKAGTSSLTECVLNKATNVAHWTTPSLKCIRDPALVHQRPAPPS

SEQ ID NO: 3 - protein, 114 aa, synthetic construct
NWVNVISDLKKIEDLIQSMHIDATLYTESDVHPSCKVTAMKCFLLELQVISLESGDASIHDTVENLIILANDSLSSNGNVTESGCKECEELEEKNIKEFLQSFVHIVQMFINTS

SEQ ID NO: 4 - protein, 297 aa, synthetic construct
ITCPPPMSVEHADIWVKSYSLYSRERYICNSGFKRKAGTSSLTECVLNKATNVAHWTTPSLKCIREPKSCDKTHTCPPCPAPELLGGPSVFLFPPKPKDTLMISRTPEVTCVVVDVSHEDPEVKFNWYVDGVEVHNAKTKPREEQYNSTYRVVSVLTVLHQDWLNGKEYKCKVSNKALPAPIEKTISKAKGQPREPQVYTLPPSRDELTKNQVSLTCLVKGFYPSDIAVEWESNGQPENNYKTTPPVLDSDGSFFLYSKLTVDKSRWQQGNVFSCSVMHEALHNHYTQKSLSLSPGK

SEQ ID NO: 5 - protein, 114 aa, synthetic construct
NWVNVISDLKKIEDLIQSMHIDATLYTESDVHPSCKVTAMKCFLLELQVISCESGDASIHDTVENLIILANNSLSSNGNVTESGCKECEELEEKNIKEFLQSFVHIVQMFINTS

SEQ ID NO: 6 - protein, 328 aa, synthetic construct
ITCPPPMSVEHADIWVKSYSLYSRERYICNSGFKRKAGTCSLTECVLNKATNVAHWTTPSLKCIRDPALVHQRPAPPSGGSGGGGSGGGSGGGGSLQEPKSSDKTHTCPPCPAPELLGGPSVFLFPPKPKDTLMISRTPEVTCWVDVSHEDPEVKFNWYVDGVEVHNAKTKPREEQYNSTYRVVSVLTVLHQDWLNGKEYKCKVSNKALPAPIEKTISKAKGQPREPQVYTLPPSREEMTKNQVSLTCLVKGFYPSDIAVEWESNGQPENNYKTTPPVLDSDGSFFLYSKLTVDKSRWQQGNVFSCSVMHEALHNHYTQKSLSLSPGK

SEQ ID NO: 7 - protein, 354 aa, synthetic construct
NWVNVISDLKKIEDLIQSMHIDATLYTESDVHPSCKVTAMKCFLLELQVISLESGDASIHDTVENLIILANNSLSSNGNVTESGCKECEELEEKNIKEFLQSFVHIVQMFINTSGGGGSGGGGSEPKSSDKTHTCPPCPAPELLGGPSVFLFPPKPKDTLMISRTPEVTCVWDVSHEDPEVKFNWYVDGVEVHNAKTKPREEQYNSTYRWSVLTVLHQDWLNGKEYKCKVSNKALPAPIEKTISKAKGQPREPQVYTLPPSREEMTKNQVSLYCLVKGFYPSDIAVEWESNGQPENNYKTTPPVLDSDGSFFLYSKLTVDKSRWQQGNVFSCSVMHEALHNHYTQKSLSLSPGK

SEQ ID NO: 8 - protein, 324 aa, synthetic construct
ITCPPPMSVEHADIWVKSYSLYSRERYICNSGFKRKAGTSSLTECVLNKATNVAHWTTPSLKCIRDPALVHQRSGGSGGGGSGGGSGGGGSLQEPKSSDKTHTCPPCPAPELLGGPSVFLFPPKPKDTLMISRTPEVTCVWDVSHEDPEVKFNWYVDGVEVHNAKTKPREEQYNSTYRVVSVLTVLHQDWLNGKEYKCKVSNKALPAPIEKTISKAKGQPREPQVYTLPPSREEMTKNQVSLTCLVKGFYPSDIAVEWESNGQPENNYKTTPPVLDSDGSFFLTSKLTVDKSRWQQGNVFSCSVMHEALHNHYTQKSLSLSPGK

SEQ ID NO: 9 - protein, 229 aa, synthetic construct
ESKYGPPCPPCPAPEFLGGPSVFLFPPKPKDTLMISRTPEVTCVVVDVSQEDPEVQFNWYVDGVEVHNAKTKPREEQFNSTYRVVSVLTVLHQDWLNGKEYKCKVSNKGLPSSIEKTISKAKGQPREPQVYTLPPSQEEMTKNQVSLWCLVKGFYPSDIAVEWESNGQPENNYKTTPPVLDSDGSFFLYSRLTVDKSRWQEGNVFSCSVMHEALHNHYTQKSLSLSLGK

SEQ ID NO: 10 - protein, 229 aa, synthetic construct
ESKYGPPCPPCPAPEFLGGPSVFLFPPKPKDTLMISRTPEVTCVVVDVSQEDPEVQFNWYVDGVEVHNAKTKPREEQFNSTYRVVSVLTVLHQDWLNGKEYKCKVSNKGLPSSIEKTISKAKGQPREPQVYTLPPSQEEMTKNQVSLSCAVKGFYPSDIAVEWESNGQPENNYKTTPPVLDSDGSFFLVSRLTVDKSRWQEGNVFSCSVMHEALHNHYTQKSLSLSLGK

SEQ ID NO: 11 - protein, 358 aa, synthetic construct
NWVNVISDLKKIEDLIQSMHIDATLYTESDVHPSCKVTAMKCFLLELQVISLESGDASIHDTVENLIILANNSLSSNGNVTESGCKECEELEEKNIKEFLQSFVHIVQMFINTSGGGGSGGGGSGGGGSESKYGPPCPPCPAPEFLGGPSVFLFPPKPKDTLMISRTPEVTCVVVDVSQEDPEVQFNWYVDGVEVHNAKTKPREEQFNSTYRVVSVLTVLHQDWLNGKEYKCKVSNKGLPSSIEKTISKAKGQPREPQVYTLPPSQEEMTKNQVSLSCAVKGFYPSDIAVEWESNGQPENNYKTTPPVLDSDGSFFLVSRLTVDKSRWQEGNVFSCSVMHEALHNHYTQKSLSLSLGK

SEQ ID NO: 12 - protein, 358 aa, synthetic construct
NWVNVISDLKKIEDLIQSMHIDATLYTESDVHPSCKVTAMKCFLLELQVISLESGDASIHDTVENLIILANDSLSSNGNVTESGCKECEELEEKNIKEFLQSFVHIVQMFINTSGGGGSGGGGSGGGGSESKYGPPCPPCPAPEFLGGPSVFLFPPKPKDTLMISRTPEVTCVVVDVSQEDPEVQFNWYVDGVEVHNAKTKPREEQFNSTYRVVSVLTVLHQDWLNGKEYKCKVSNKGLPSSIEKTISKAKGQPREPQVYTLPPSQEEMTKNQVSLSCAVKGFYPSDIAVEWESNGQPENNYKTTPPVLDSDGSFFLVSRLTVDKSRWQEGNVFSCSVMHEALHNHYTQKSLSLSLGK

SEQ ID NO: 13 - protein, 358 aa, synthetic construct
NWVNVISDLKKIEDLIQSMHIDATLYTESDVHPSCKVTAMKCFLEELQVISEESGDASIHDTVENLIILANDSLSSNGNVTESGCKECEELEEKNIKEFLQSFVHIVQMFINTSGGGGSGGGGSGGGGSESKYGPPCPPCPAPEFLGGPSVFLFPPKPKDTLMISRTPEVTCVVVDVSQEDPEVQFNWYVDGVEVHNAKTKPREEQFNSTYRVVSVLTVLHQDWLNGKEYKCKVSNKGLPSSIEKTISKAKGQPREPQVYTLPPSQEEMTKNQVSLSCAVKGFYPSDIAVEWESNGQPENNYKTTPPVLDSDGSFFLVSRLTVDKSRWQEGNVFSCSVMHEALHNHYTQKSLSLSLGK

SEQ ID NO: 14 - protein, 358 aa, synthetic construct
NWVNVISDLKKIEDLIQSMHIDATLYTESDVHPSCKVTAMKCFLDELQVISDESGDASIHDTVENLIILANDSLSSNGNVTESGCKECEELEEKNIKEFLQSFVHIVQMFINTSGGGGSGGGGSGGGGSSEKYGPPCPPCPAPEFLGGPSVFLFPPKPKDTLMISRTPEVTCVVVDVSQEDPEVQFNWYVDGVEVHNAKTKPREEQFNSTYRVVSVLTVLHQDWLNGKEYKCKVSNKGLPSSIEKTISKAKGQPREPQVYTLPPSQEEMTKNQVSLWCLVKGFYPSDIAVEWESNGQPENNYKTTPPVLDSDGSFFLYSRLTVDKSRWQEGNVFSCSVMHEALHNHYTQKSLSLSLGK

SEQ ID NO: 15 - protein, 355 aa, synthetic construct
NWVNVISDLKKIEDLIQSMHIDATLYTESDVHPSCKVTAMKCFLLELQVISLESGDASIHDTVENLIILANDSLSSNGNVTESGCKECEELEEKNIKEFLQSFVHIVQMFIGGGGSGGGGSGGGGSESKYGPPCPPCPAPEFLGGPSVFLFPPKPKDTLMISRTPEVTCVVVDVSQEDPEVQFNWYVDGVEVHNAKTKPREEQFNSTYRVVSVLTVLHQDWLNGKEYKCKVSNKGLPSSIEKTISKAKGQPREPQVYTLPPSQEEMTKNQVSLSCAVKGFYPSDIAVEWESNGQPENNYKTTPPVLDSDGSFFLVSRLTVDKSRWQEGNVFSCSVMHEALHNHYTQKSLSLSLGK

SEQ ID NO: 16 - protein, 358 aa, synthetic construct
NWVNVISDLKKIEDLIQSMHIDATLYTESDVHPSCKVTAMKCFLDELQVISEESGDASIHDTVENLIILANDSLSSNGNVTESGCKECEELEEKNIKEFLQSFVHIVQMFINTSGGGGSGGGGSGGGGSESKYGPPCPPCPAPEFLGGPSVFLFPPKPKDTLMISRTPEVTCVVVDVSQEDPEVQFNWYVDGVEVHNAKTKPREEQFNSTYRVVSVLTVLHQDWLNGKEYKCKVSNKGLPSSIEKTISKAKGQPREPQVYTLPPSQEEMTKNQVSLSCAVKGFYPSDIAVEWESNGQPENNYKTTPPVLDSDGSFFLVSRLTVDKSRWQEGNVFSCSVMHEALHNHYTQKSLSLSLGK

SEQ ID NO: 17 - protein, 358 aa, synthetic construct
NWVNVISDLKKIEDLIQSMHIDATLYTESDVHPSCKVTAMKCFLEELQVISDESGDASIHDTVENLIILANDSLSSNGNVTESGCKECEELEEKNIKEFLQSFVHIVQMFINTSGGGGSGGGGSGGGGSESKYGPPCPPCPAPEFLGGPSVFLFPPKPKDTLMISRTPEVTCVVVDVSQEDPEVQFNWYVDGVEVHNAKTKPREEQFNSTYRVVSVLTVLHQDWLNGKEYKCKVSNKGLPSSIEKTISKAKGQPREPQVYTLPPSQEEMTKNQVSLSCAVKGFYPSDIAVEWESNGQPENNYKTTPPVLDSDGSFFLVSRLTVDKSRWQEGNVFSCSVMHEALHNHYTQKSLSLSLGK

SEQ ID NO: 18 - protein, 355 aa, synthetic construct
NWVNVISDLKKIEDLIQSMHIDATLYTESDVHPSCKVTAMKCFLDELQVISDESGDASIHDTVENLIILANDSLSSNGNVTESGCKECEELEEKNIKEFLQSFVHIVQMFIGGGGSGGGGSGGGGSESKYGPPCPPCPAPEFLGGPSVFLFPPKPKDTLMISRTPEVTCVVVDVSQEDPEVQFNWYVDGVEVHNAKTKPREEQFNSTYRVVSVLTVLHQDWLNGKEYKCKVSNKGLPSSIEKTISKAKGQPREPQVYTLPPSQEEMTKNQVSLSCAVKGFYPSDIAVEWESNGQPENNYKTTPPVLDSDGSFFLVSRLTVDKSRWQEGNVFSCSVMHEALHNHYTQKSLSLSLGK

SEQ ID NO: 19 - protein, 307 aa, synthetic construct
ITCPPPMSVEHADIWVKSYSLYSRERYICNSGFKRKAGTSSLTECVLNKATNVAHWTTPSLKCIRDPALVHQRPAPPSESKYGPPCPPCPAPEFLGGPSVFLFPPKPKDTLMISRTPEVTCVVVDVSQEDPEVQFNWYVDGVEVHNAKTKPREEQFNSTYRVVSVLTVLHQDWLNGKEYKCKVSNKGLPSSIEKTISKAKGQPREPQVYTLPPSQEEMTKNQVSLWCLVKGFYPSDIAVEWESNGQPENNYKTTPPVLDSDGSFFLYSRLTVDKSRWQEGNVFSCSVMHEALHNHYTQKSLSLSLGK

SEQ ID NO: 20 - protein, 322 aa, synthetic construct
ITCPPPMSVEHADIWVKSYSLYSRERYICNSGFKRKAGTSSLTECVLNKATNVAHWTTPSLKCIRDPALVHQRPAPPSGGGGSGGGGSGGGGSESKYGPPCPPCPAPEFLGGPSVFLFPPKPKDTLMISRTPEVTCVVVDVSQEDPEVQFNWYVDGVEVHNAKTKPREEQFNSTYRVVSVLTVLHQDWLNGKEYKCKVSNKGLPSSIEKTISKAKGQPREPQVYTLPPSQEEMTKNQVSLWCLVKGFYPSDIAVEWESNGQPENNYKTTPPVLDSDGSFFLYSRLTVDKSRWQEGNVFSCSVMHEALHNHYTQKSLSLSLGK

SEQ ID NO: 21 - DNA, 342 bp, synthetic construct
  source 1..342: mol_type = other DNA
aactgggtaaatgtgatcagcgacttgaagaagatcgaagacctcattcaatcaatgcacatcgacgctacactgtatactgaaagcgatgttcacccaagttgcaaggtgactgccatgaagtgttttctgctggagctccaagttattagtctggagagcggtgacgcctcaattcacgacaccgtcgaaaacctgatcattctggccaacgactccctgtcttcaaacggcaacgtgacagagtccggatgtaaagagtgcgaggagctggaggagaagaacattaaagaatttctgcagagcttcgtgcacatcgtccagatgtttatcaatacctct

SEQ ID NO: 22 - DNA, 891 bp, synthetic construct
  source 1..891: mol_type = other DNA
ataacatgtcctcccccaatgtctgtggaacatgccgatatctgggtgaagagctactccctttacagtagagagagatacatctgcaattcagggttcaagcgaaaagccgggactagttccctcaccgagtgtgtgttgaacaaggctacaaacgtggctcactggaccacccctagtctcaagtgtatacgggagccaaagtcttgcgataagacccacacttgtcctccctgccctgcccctgaattgcttggcggaccaagtgtgttcctgtttccacccaaacccaaagatacccttatgattagccgcacccccgaggtcacctgtgtcgttgtggatgtctcacatgaggatcctgaggtcaagtttaactggtacgtggacggcgtggaggtgcacaatgcaaaaactaagccccgcgaagagcagtataactctacttaccgagtggtgagcgtgctcactgtgcttcaccaggattggctgaatgggaaagagtacaagtgcaaggtctctaacaaagccttgcctgctccaatcgagaagacaatcagcaaggctaagggtcagccaagggaaccccaagtttacaccctgccaccctctagagacgagctgaccaagaaccaggtgtcattgacctgccttgttaagggcttctacccttccgacattgctgtggagtgggaatcaaatggccagcctgaaaacaactataaaacaacacccccagtcttggactctgacgggagtttcttcctttatagcaaactcactgtggataaaagtcgatggcagcagggaaacgtcttttcttgttccgtcatgcatgaggctttgcataatcattacacccagaaatccctcagtctgtcccctggcaag

SEQ ID NO: 23 - DNA, 342 bp, synthetic construct
  source 1..342: mol_type = other DNA
aattgggtcaacgtgatctctgaccttaaaaaaattgaagacctgatccagtcaatgcacattgacgctacactctacacagagtccgatgtgcaccctagctgtaaagtgactgccatgaaatgcttcctcctggagctgcaggtcatatcatgcgaaagcggagatgctagcatccacgacaccgtggagaacctgataatattggctaataacagtctgtctagtaacggcaacgtgacagaaagcggctgcaaggaatgtgaagaactggaagagaagaacatcaaggagttcttgcaatcattcgtgcacattgtccagatgtttatcaacacgagc

SEQ ID NO: 24 - DNA, 987 bp, synthetic construct
  source 1..987: mol_type = other DNA
atcacctgtcccccccctatgtctgtggagcacgctgacatctgggtgaaatcctattctctgtactctagggagcgctacatctgtaactccggcttcaagcggaaggccggtacttgcagcctgacagagtgtgtgctgaataaggcaaccaacgtggcccactggaccacacctagtctgaagtgtatcagggatcccgccctggtgcaccagaggcccgctcccccaagcggcggcagtggcggaggaggctccggcggcggttctggcggcggcggatctctgcaggaaccaaagagctccgataaaacccacacctgccctccctgccctgctcccgagctgctaggcggaccatctgtgttcctgtttccccccaagcccaaggacaccctgatgatctccagaacacctgaggtgacctgttgggtggacgtgagccatgaggacccagaagtgaagttcaactggtacgtggacggagtggaggtgcacaatgctaagactaagcctcgggaggagcagtacaatagcacctatcgggtggtgagcgtgctgactgtgcttcatcaggactggctgaacggaaaggagtacaagtgtaaggtgtctaacaaggccctgcccgcccccatcgagaagacaatctctaaggccaaaggccagcctcgagagccacaggtgtacacactgccccccagccgggaggagatgaccaagaatcaggtgagcctgacctgtctggtgaaaggcttttacccaagcgacatcgctgtggagtgggaatctaacggccagcctgagaacaactacaaaaccacccctcctgtgctcgactccgacggctcctttttcctgtactccaagctgacagtcgacaagtctcgatggcagcagggcaatgtcttctcttgttccgtgatgcacgaagccctgcacaaccactatacccagaaaagcctgtccctgtcccccggcaagtga

SEQ ID NO: 25 - DNA, 1065 bp, synthetic construct
  source 1..1065: mol_type = other DNA
aactgggtgaacgtgatctctgacctgaagaagattgaggacctgatccagtctatgcacatcgacgccaccctgtacaccgagtccgacgtccacccttcctgtaaggtgacagccatgaagtgcttcctgctggagctgcaggtgatctccctggagtccggggacgccagcatccatgataccgtggaaaacctgatcattctggccaacaactctctgagctccaatggcaacgtgaccgagagcggctgcaaggagtgcgaggaactggaggagaagaacatcaaggagtttctgcagtccttcgtccatatcgtgcagatgttcattaacacatccggcggcggcggctccggcggcggcgggtctgagcctaagagttccgacaagacccacacctgccccccctgcccagcccctgagctgctgggtggaccatccgtgttcctgttcccacccaagcctaaggataccctgatgatctctcgcacaccagaggtgacctgcgtgtgggacgtgagccacgaggatcccgaggtgaagttcaactggtacgtggacggggtggaggtgcataacgctaagaccaaaccaagagaggaacagtataatagtacataccgttggtctgtgctgacagtgcttcaccaggactggctgaacggaaaggagtacaagtgcaaggtgagcaataaggctctgcctgcccccatcgagaagactatctctaaggccaagggccagccccgggagcctcaggtgtacacactgccccctagcagagaggagatgacaaagaaccaggtgtccctgtattgtctggtgaaaggattctaccccagcgacatcgcagtggaatgggagtctaacgggcagccagagaacaattataagactaccccacccgtgctggacagcgacggatcattcttcctgtactctaagctcactgtggacaagagccgttggcagcaggggaacgtgttttcctgcagtgtgatgcacgaggctctgcacaatcactacacccagaagtctctgtccctgtctcccggcaagtga

SEQ ID NO: 26 - DNA, 975 bp, synthetic construct
  source 1..975: mol_type = other DNA
atcacatgtccccccccaatgtctgtggagcacgccgacatttgggtgaaaagctactctctgtactcccgggagagatacatctgtaactccggtttcaagaggaaggccggcaccagctctctgacagagtgcgtcctgaataaggcaaccaatgttgctcattggaccactccatctctgaagtgtatccgggaccccgccctggtgcatcagagatccggcggctccggaggcggcggcagcggaggtggctctggaggcggcggctccctgcaggaaccaaaatctagcgataagacacacacctgtcccccttgccccgcccccgagttgctgggcggcccatctgtgttcctgtttcctccaaagccaaaggacaccctgatgatttctcggaccccagaggtgacctgtgtctgggatgtgagccacgaggaccccgaggtgaagttcaactggtacgtggacggcgtggaggtgcacaatgccaagaccaagcctcgcgaggagcagtataacagcacctaccgggtggtgagcgtcctgaccgtgctgcatcaggactggctgaatggaaaggagtacaaatgcaaggtgtcaaacaaggccctgccagctccaatcgaaaagaccatcagcaaggccaagggccagccccgcgagccacaggtgtacaccctgcccccctccagagaggagatgactaagaaccaggtgtccctgacatgcctggtgaagggcttttacccatccgatattgctgtggagtgggagtccaacggccagcctgagaacaactacaagaccacacctcctgtgctggattctgatggctcctttttcctgaccagcaagctgaccgtggacaagtctcggtggcagcagggcaacgtgttctcttgctccgtgatgcacgaggctctgcacaaccattacacacagaagtccctctccttgagccccggcaagtga

SEQ ID NO: 27 - DNA, 1077 bp, synthetic construct
  source 1..1077: mol_type = other DNA
aactgggtgaacgtgatctctgacctgaagaaaatcgaggacctgatccagtcaatgcacatcgatgccaccctgtacacagagtcagatgtgcaccctagctgcaaggtcaccgctatgaaatgtttcctgctggagctgcaggtgatcagcctggagtcaggcgacgccagcatccacgataccgtggagaacctgatcatcctggctaacaactctctgtcctccaacggaaacgtgaccgagagtggctgcaaggagtgtgaggaactggaggagaagaacatcaaggagtttctgcagtcctttgtgcatatcgtgcagatgttcattaacacatctggggggggcggcagcggcggcgggggcagtggcggcggtggttctgaatccaaatacgggccaccctgccccccttgccccgcccctgaattcttgggaggccccagtgtgttcctgttcccccccaagcctaaggacactctgatgatctctcgcaccccagaggtgacctgtgtggtggtggacgtgtctcaggaagatcccgaggtccagttcaactggtacgtggacggagtggaggtgcacaacgccaaaaccaagccacgcgaggagcagttcaactccacctatagggtggtgtccgttctgaccgtgctgcaccaggattggctgaatggcaaagaatacaagtgcaaggtgagcaacaagggcctgccttctagtatcgagaagactatctccaaggccaagggccagcccagagagcctcaggtgtataccctgccaccatctcaggaggagatgaccaagaaccaggtgagcctgagctgtgcagtgaaaggcttttatccttccgacatcgctgtggaatgggagtccaacggccagcccgagaataactataagacaacccctcctgtgctggacagcgacggctcattcttcctggtgtccaggctgaccgtggacaagtctcggtggcaggagggaaatgtgttcagttgctccgtgatgcacgaggctctgcacaaccactatacccagaagtctctttctctgtccctgggcaagtga

SEQ ID NO: 28 - DNA, 1077 bp, synthetic construct
  source 1..1077: mol_type = other DNA
aactgggtgaacgtgatctctgacctgaagaaaatcgaggacctgatccagtcaatgcacatcgatgccaccctgtacacagagtcagatgtgcaccctagctgcaaggtcaccgctatgaaatgtttcctgctggagctgcaggtgatcagcctggagtcaggcgacgccagcatccacgataccgtggagaacctgatcatcctggctaacgactctctgtcctccaacggaaacgtgaccgagagtggctgcaaggagtgtgaggaactggaggagaagaacatcaaggagtttctgcagtcctttgtgcatatcgtgcagatgttcattaacacatctggggggggcggcagcggcggcgggggcagtggcggcggtggttctgaatccaaatacgggccaccctgccccccttgccccgcccctgaattcttgggaggccccagtgtgttcctgttcccccccaagcctaaggacactctgatgatctctcgcaccccagaggtgacctgtgtggtggtggacgtgtctcaggaagatcccgaggtccagttcaactggtacgtggacggagtggaggtgcacaacgccaaaaccaagccacgcgaggagcagttcaactccacctatagggtggtgtccgttctgaccgtgctgcaccaggattggctgaatggcaaagaatacaagtgcaaggtgagcaacaagggcctgccttctagtatcgagaagactatctccaaggccaagggccagcccagagagcctcaggtgtataccctgccaccatctcaggaggagatgaccaagaaccaggtgagcctgagctgtgcagtgaaaggcttttatccttccgacatcgctgtggaatgggagtccaacggccagcccgagaataactataagacaacccctcctgtgctggacagcgacggctcattcttcctggtgtccaggctgaccgtggacaagtctcggtggcaggagggaaatgtgttcagttgctccgtgatgcacgaggctctgcacaaccactatacccagaagtctctttctctgtccctgggcaagtga

SEQ ID NO: 29 - DNA, 1077 bp, synthetic construct
  source 1..1077: mol_type = other DNA
aactgggtgaacgtgatctctgacctgaagaaaatcgaggacctgatccagtcaatgcacatcgatgccaccctgtacacagagtcagatgtgcaccctagctgcaaggtcaccgctatgaaatgtttcctggaggagctgcaggtgatcagcgaggagtcaggcgacgccagcatccacgataccgtggagaacctgatcatcctggctaacgactctctgtcctccaacggaaacgtgaccgagagtggctgcaaggagtgtgaggaactggaggagaagaacatcaaggagtttctgcagtcctttgtgcatatcgtgcagatgttcattaacacatctggggggggcggcagcggcggcgggggcagtggcggcggtggttctgaatccaaatacgggccaccctgccccccttgccccgcccctgaattcttgggaggccccagtgtgttcctgttcccccccaagcctaaggacactctgatgatctctcgcaccccagaggtgacctgtgtggtggtggacgtgtctcaggaagatcccgaggtccagttcaactggtacgtggacggagtggaggtgcacaacgccaaaaccaagccacgcgaggagcagttcaactccacctatagggtggtgtccgttctgaccgtgctgcaccaggattggctgaatggcaaagaatacaagtgcaaggtgagcaacaagggcctgccttctagtatcgagaagactatctccaaggccaagggccagcccagagagcctcaggtgtataccctgccaccatctcaggaggagatgaccaagaaccaggtgagcctgagctgtgcagtgaaaggcttttatccttccgacatcgctgtggaatgggagtccaacggccagcccgagaataactataagacaacccctcctgtgctggacagcgacggctcattcttcctggtgtccaggctgaccgtggacaagtctcggtggcaggagggaaatgtgttcagttgctccgtgatgcacgaggctctgcacaaccactatacccagaagtctctttctctgtccctgggcaagtga

SEQ ID NO: 30 - DNA, 1077 bp, synthetic construct
  source 1..1077: mol_type = other DNA
aattgggtgaacgtgatctccgacctgaagaaaatcgaggatctgatccagtccatgcacatcgacgccaccctgtacaccgaatctgacgtgcacccatcttgtaaggtgaccgctatgaaatgctttctggacgaactgcaggtgatttccgacgagtccggtgacgcctccatccacgataccgtggaaaacctgatcattctggctaacgattccctgtctagcaacggaaacgtgaccgagagcggatgtaaagagtgcgaggagctggaggaaaagaacatcaaggaatttctgcagagcttcgtgcacatcgtgcagatgttcatcaatacatcaggcggcggcggcagcgggggcggcggctcaggcggcggcggcagcgagtccaagtacggacccccctgcccaccctgccccgctcccgagttcctgggcggcccaagcgtgtttctgtttcctcccaagcccaaagacacactgatgatctctaggacccccgaggtgacatgcgtagtggtggacgtgtctcaggaggatccagaggtccagttcaactggtacgtggacggtgtggaagtgcacaacgctaagaccaagcctcgcgaggagcagtttaacagtacctaccgggtggtgtccgtgctgactgtgctgcaccaggactggctgaatggcaaggagtataagtgcaaggtgtccaacaaaggactgccttctagcatcgagaagaccatcagtaaggccaagggccagccaagggagccacaggtttacacactgcccccaagccaggaggagatgaccaagaaccaggtgtcactgtggtgcctggtgaaaggcttttacccttccgacatcgccgtggagtgggagagcaatggacagcctgagaacaactacaagactaccccccctgttctggactccgatggctcctttttcctgtattccaggctgactgtggacaagtccaggtggcaggaggggaatgtgttcagttgtagcgtgatgcacgaggccctgcataaccattatacccagaagtctcttagcctgagcctgggcaagtga

SEQ ID NO: 31 - DNA, 1068 bp, synthetic construct
  source 1..1068: mol_type = other DNA
aactgggtgaatgtgatctccgatctgaagaagatcgaggatctgatccagtccatgcacatcgatgccaccctgtatacagagtccgacgtgcacccctcctgcaaggtgactgcaatgaagtgcttcctgctggaactgcaggtgatcagcctggagtccggcgatgcatcaatccacgacacagtggagaatctgatcattctggccaacgacagcctgtcctccaacggaaacgtgacagagagcggctgcaaggagtgtgaggagctggaagagaagaacatcaaggagttcctgcagtctttcgtgcacatcgtgcagatgttcatcggcggcgggggaagcggcggcggcgggagcggcggaggcggaagcgagagcaagtacggccctccatgccccccatgtcccgcccctgaatttctgggagggccttctgtgttcctgttccccccaaagccaaaggacaccctgatgatttcccgaactcctgaggtcacctgcgtggtggtggatgtgagtcaggaagacccagaggtgcagttcaactggtatgtggacggggtggaagtgcataacgccaaaaccaagccacgggaggagcagttcaactctacctatagggtggtgagcgtgctcaccgtgctgcaccaggactggctgaatggcaaagagtacaagtgcaaggtgtccaataagggcctgcctagcagcatcgagaagaccatttcaaaggctaagggccagcccagggaaccacaggtgtacaccctgcccccctctcaggaagaaatgactaagaaccaggtgagcctgtcctgcgctgtgaagggcttctacccatccgacatcgccgtggaatgggagagcaacgggcagccagagaataactacaaaactacccctcccgtcctggacagcgacggcagtttctttctggtcagccggctgaccgtggacaagtccaggtggcaggagggcaatgtgttctcttgctccgtgatgcatgaggccctgcataatcactacacacagaagagcctgtctctgtctctgggtaagtga

SEQ ID NO: 32 - DNA, 1077 bp, synthetic construct
  source 1..1077: mol_type = other DNA
aactgggtgaacgtgatctctgacctgaagaaaatcgaggacctgatccagtcaatgcacatcgatgccaccctgtacacagagtcagatgtgcaccctagctgcaaggtcaccgctatgaaatgtttcctggacgagctgcaggtgatcagcgaggagtcaggcgacgccagcatccacgataccgtggagaacctgatcatcctggctaacgactctctgtcctccaacggaaacgtgaccgagagtggctgcaaggagtgtgaggaactggaggagaagaacatcaaggagtttctgcagtcctttgtgcatatcgtgcagatgttcattaacacatctggggggggcggcagcggcggcgggggcagtggcggcggtggttctgaatccaaatacgggccaccctgccccccttgccccgcccctgaattcttgggaggccccagtgtgttcctgttcccccccaagcctaaggacactctgatgatctctcgcaccccagaggtgacctgtgtggtggtggacgtgtctcaggaagatcccgaggtccagttcaactggtacgtggacggagtggaggtgcacaacgccaaaaccaagccacgcgaggagcagttcaactccacctatagggtggtgtccgttctgaccgtgctgcaccaggattggctgaatggcaaagaatacaagtgcaaggtgagcaacaagggcctgccttctagtatcgagaagactatctccaaggccaagggccagcccagagagcctcaggtgtataccctgccaccatctcaggaggagatgaccaagaaccaggtgagcctgagctgtgcagtgaaaggcttttatccttccgacatcgctgtggaatgggagtccaacggccagcccgagaataactataagacaacccctcctgtgctggacagcgacggctcattcttcctggtgtccaggctgaccgtggacaagtctcggtggcaggagggaaatgtgttcagttgctccgtgatgcacgaggctctgcacaaccactatacccagaagtctctttctctgtccctgggcaagtga

SEQ ID NO: 33 - DNA, 1077 bp, synthetic construct
  source 1..1077: mol_type = other DNA
aattgggtgaacgtgatctccgacctgaagaaaatcgaggatctgatccagtccatgcacatcgacgccaccctgtacaccgaatctgacgtgcacccatcttgtaaggtgaccgctatgaaatgctttctggaagaactgcaggtgatttccgacgagtccggtgacgcctccatccacgataccgtggaaaacctgatcattctggctaacgattccctgtctagcaacggaaacgtgaccgagagcggatgtaaagagtgcgaggagctggaggaaaagaacatcaaggaatttctgcagagcttcgtgcacatcgtgcagatgttcatcaatacatcaggcggcggcggcagcgggggcggcggctcaggcggcggcggcagcgagtccaagtacggacccccctgcccaccctgccccgctcccgagttcctgggcggcccaagcgtgtttctgtttcctcccaagcccaaagacacactgatgatctctaggacccccgaggtgacatgcgtagtggtggacgtgtctcaggaggatccagaggtccagttcaactggtacgtggacggtgtggaagtgcacaacgctaagaccaagcctcgcgaggagcagtttaacagtacctaccgggtggtgtccgtgctgactgtgctgcaccaggactggctgaatggcaaggagtataagtgcaaggtgtccaacaaaggactgccttctagcatcgagaagaccatcagtaaggccaagggccagccaagggagccacaggtttacacactgcccccaagccaggaggagatgaccaagaaccaggtgtcactgtcctgcgctgtgaaaggcttttacccttccgacatcgccgtggagtgggagagcaatggacagcctgagaacaactacaagactaccccccctgttctggactccgatggctcctttttcctggtgtccaggctgactgtggacaagtccaggtggcaggaggggaatgtgttcagttgtagcgtgatgcacgaggccctgcataaccattatacccagaagtctcttagcctgagcctgggcaagtga

SEQ ID NO: 34 - DNA, 1068 bp, synthetic construct
  source 1..1068: mol_type = other DNA
aactgggtgaatgtgatctccgatctgaagaagatcgaggatctgatccagtccatgcacatcgatgccaccctgtatacagagtccgacgtgcacccctcctgcaaggtgactgcaatgaagtgcttcctggatgaactgcaggtgatcagcgatgagtccggcgatgcatcaatccacgacacagtggagaatctgatcattctggccaacgacagcctgtcctccaacggaaacgtgacagagagcggctgcaaggagtgtgaggagctggaagagaagaacatcaaggagttcctgcagtctttcgtgcacatcgtgcagatgttcatcggcggcgggggaagcggcggcggcgggagcggcggaggcggaagcgagagcaagtacggccctccatgccccccatgtcccgcccctgaatttctgggagggccttctgtgttcctgttccccccaaagccaaaggacaccctgatgatttcccgaactcctgaggtcacctgcgtggtggtggatgtgagtcaggaagacccagaggtgcagttcaactggtatgtggacggggtggaagtgcataacgccaaaaccaagccacgggaggagcagttcaactctacctatagggtggtgagcgtgctcaccgtgctgcaccaggactggctgaatggcaaagagtacaagtgcaaggtgtccaataagggcctgcctagcagcatcgagaagaccatttcaaaggctaagggccagcccagggaaccacaggtgtacaccctgcccccctctcaggaagaaatgactaagaaccaggtgagcctgtcctgcgctgtgaagggcttctacccatccgacatcgccgtggaatgggagagcaacgggcagccagagaataactacaaaactacccctcccgtcctggacagcgacggcagtttctttctggtcagccggctgaccgtggacaagtccaggtggcaggagggcaatgtgttctcttgctccgtgatgcatgaggccctgcataatcactacacacagaagagcctgtctctgtctctgggtaagtga

SEQ ID NO: 35 - protein, 924 aa, synthetic construct
ATCACTTGTCCACCACCCATGTCCGTGGAGCACGCCGATATCTGGGTGAAGAGCTACAGCCTGTACAGCCGAGAACGCTACATCTGTAACTCCGGCTTCAAGAGAAAGGCTGGCACTAGCTCTCTGACCGAGTGCGTGCTCAACAAGGCAACCAACGTGGCCCACTGGACCACACCTTCCCTGAAGTGTATTCGGGATCCTGCTCTGGTGCACCAGCGGCCCGCCCCTCCATCAGAGTCAAAGTACGGCCCCCCATGTCCACCATGCCCTGCACCTGAGTTTCTGGGCGGCCCCTCCGTGTTTCTGTTTCCCCCCAAGCCTAAGGACACTCTGATGATTTCAAGGACCCCAGAGGTGACCTGCGTGGTCGTGGACGTGAGCCAGGAGGACCCAGAGGTGCAGTTTAATTGGTACGTGGACGGCGTGGAGGTGCATAATGCTAAGACCAAACCTCGGGAGGAGCAGTTCAACTCTACCTACCGGGTGGTGAGCGTGCTGACCGTCCTGCACCAGGATTGGCTGAATGGCAAGGAGTACAAGTGCAAAGTGTCCAATAAGGGCCTGCCTAGCTCCATCGAGAAAACTATCTCCAAAGCCAAGGGCCAGCCTCGGGAACCACAGGTGTACACCCTGCCCCCTAGCCAGGAAGAAATGACTAAGAACCAGGTGTCTCTGTGGTGTCTGGTGAAGGGCTTCTACCCTAGCGATATCGCCGTGGAGTGGGAGTCCAACGGCCAGCCCGAGAACAATTACAAGACTACTCCCCCCGTGCTGGACTCTGACGGATCCTTCTTTCTGTACTCTAGACTGACCGTGGACAAGAGCCGGTGGCAGGAGGGCAATGTGTTCTCTTGCTCAGTGATGCACGAGGCTCTGCACAACCACTACACCCAGAAGTCTCTGAGTCTCAGCCTGGGAAAGTGA

SEQ ID NO: 36 - protein, 969 aa, synthetic construct
ATTACCTGCCCCCCTCCCATGAGTGTGGAGCACGCAGATATCTGGGTCAAAAGCTACTCCCTGTATTCTCGGGAACGGTATATTTGTAATTCAGGCTTTAAACGGAAGGCCGGCACATCTTCCCTGACCGAGTGCGTGCTGAACAAGGCCACTAATGTGGCTCACTGGACCACACCCTCCCTGAAATGCATCAGGGACCCTGCCCTGGTGCACCAGCGGCCCGCCCCTCCCTCTGGCGGCGGCGGCTCCGGTGGCGGCGGGAGCGGCGGCGGCGGCAGCGAGAGCAAGTACGGCCCCCCTTGCCCTCCCTGCCCCGCACCTGAGTTTCTGGGCGGACCCTCTGTGTTCCTGTTCCCACCCAAGCCAAAAGATACCCTGATGATCAGCCGCACACCCGAGGTGACCTGCGTGGTGGTGGACGTGTCCCAGGAGGACCCTGAGGTCCAGTTCAATTGGTACGTGGATGGCGTGGAGGTGCACAACGCTAAGACCAAGCCACGGGAAGAGCAGTTCAACAGCACCTACCGCGTGGTGAGTGTGCTGACCGTGTTGCACCAGGATTGGCTGAATGGCAAGGAGTACAAGTGTAAGGTGAGCAATAAGGGCCTGCCCTCTAGTATTGAGAAGACCATTAGCAAGGCCAAAGGGCAGCCTAGGGAGCCTCAGGTGTACACACTGCCTCCCAGCCAGGAGGAAATGACCAAGAATCAGGTGAGCCTGTGGTGCCTGGTGAAGGGCTTCTACCCCTCCGATATCGCCGTGGAGTGGGAGTCCAACGGGCAGCCTGAAAACAATTACAAGACCACCCCTCCTGTACTGGACAGCGACGGCTCCTTCTTCCTGTACTCTCGCCTGACCGTGGACAAGTCCAGATGGCAGGAGGGGAACGTGTTCTCCTGCAGCGTGATGCACGAGGCCCTGCACAACCACTATACACAGAAGTCTCTGTCTCTGAGCCTGGGCAAGTGA

SEQ ID NO: 37 - DNA, 690 bp, synthetic construct
  source 1..690: mol_type = other DNA
gagtccaagtacggccccccttgtcctccctgtcccgccccagagttcctgggaggcccctccgtgtttctgttccctcctaagccaaaggacacactgatgatctctcgcactccagaggtgacatgcgtggtggtggacgtgtctcaggaggaccccgaggtgcagtttaactggtacgtggacggcgtggaggttcacaatgctaagaccaagccccgggaagagcagtttaacagtacctatagggtggtgtccgtgctgactgtgctgcatcaggactggctgaacggcaaagagtacaagtgtaaggtgagcaacaagggcctgcccagctccatcgagaagactatctccaaagccaaaggccagcctcgggagcctcaggtgtacaccctgccacccagccaggaggagatgacaaagaaccaggtgtctctgtggtgcctggtgaagggcttctatccctccgacatcgctgtggaatgggagtccaacgggcagcccgaaaataattacaagaccacccctcccgtgctggactctgacggcagcttttttctgtatagtcggctgaccgtggataagagccggtggcaggagggcaacgtgttctcctgctcagtgatgcacgaggccctgcataaccactacactcagaagtccctgagcctgtctctcggcaagtga

SEQ ID NO: 38 - DNA, 690 bp, synthetic construct
  source 1..690: mol_type = other DNA
gagtccaagtacggccccccttgtcctccctgtcccgccccagagttcctgggaggcccctccgtgtttctgttccctcctaagccaaaggacacactgatgatctctcgcactccagaggtgacatgcgtggtggtggacgtgtctcaggaggaccccgaggtgcagtttaactggtacgtggacggcgtggaggttcacaatgctaagaccaagccccgggaagagcagtttaacagtacctatagggtggtgtccgtgctgactgtgctgcatcaggactggctgaacggcaaagagtacaagtgtaaggtgagcaacaagggcctgcccagctccatcgagaagactatctccaaagccaaaggccagcctcgggagcctcaggtgtacaccctgccacccagccaggaggagatgacaaagaaccaggtgtctctgtcttgcgccgtgaagggcttctatccctccgacatcgctgtggaatgggagtccaacgggcagcccgaaaataattacaagaccacccctcccgtgctggactctgacggcagcttttttctggtgagtcggctgaccgtggataagagccggtggcaggagggcaacgtgttctcctgctcagtgatgcacgaggccctgcataaccactacactcagaagtccctgagcctgtctctcggcaagtga

SEQ ID NO: 39 - protein, 20 aa, synthetic construct
MYSMGLASCVTLTLVLLVNS

SEQ ID NO: 40 - DNA, 60 bp, synthetic construct
  source 1..60: mol_type = other DNA
atgtacagcatgcagctcgcatcctgtgtcacattgacacttgtgctccttgtcaacagc